European Patent Application EP 4 714 969 A1, published March 25, 2026. Title: COMPOSITIONS COMPRISING sTIGIT AND PD-1/PD-L1 AXIS INHIBITORS AND USES THEREOF. Applicant: FUNDACIÓ PRIVADA INSTITUT DE RECERCA SOBRE IMMUNOPATOLOGIES - CAIXA IRSICAIXA. The sequence listing filed with the application follows.

SEQUENCE LISTING (45 sequences)

SEQ ID NO: 1 - protein, 109 aa, synthetic construct
MMTGTIETTGNISAEKGGSIILQCHLSSTTAQVTQVNWEQQDQLLAICNADLGWHISPSFKDRVAPGPGLGLTLQSLTVNDTGEYFCIYHTYPDGTYTGRIFLEVLESS

SEQ ID NO: 2 - protein, 105 aa, synthetic construct
TIDTKRNISAEEGGSVILQCHFSSDTAEVTQVDWKQQDQLLAIYSVDLGWHVASVFSDRVVPGPSLGLTFQSLTMNDTGEYFCTYHTYPGGIYKGRIFLKVQESS

SEQ ID NO: 3 - protein, 232 aa, synthetic construct
KSCDKTHTCPPCPAPELLGGPSVFLFPPKPKDTLMISRTPEVTCVVVDVSHEDPEVKFNWYVDGVEVHNAKTKPREEQYNSTYRVVSVLTVLHQDWLNGKEYKCKVSNKALPAPIEKTISKAKGQPREPQVYTLPPSRDELTKNQVSLTCLVKGFYPSDIAVEWESNGQPENNYKTTPPVLDSDGSFFLYSKLTVDKSRWQQGNVFSCSVMHEALHNHYTQKSLSLSPGKRS

SEQ ID NO: 4 - protein, 231 aa, synthetic construct
ESKYGPPCPPCPAPEFLGGPSVFLFPPKPKDTLMISRTPEVTCVVVDVSQEDPEVQFNWYVDGVEVHNAKTKPREEQFNSTYRVVSVLTVLHQDWLNGKEYKCKVSNKGLPSSIEKTISKAKGQPREPQVYTLPPSQEEMTKNQVSLTCLVKGFYPSDIAVEWESNGQPENNYKTTPPVLDSDGSFFLYSRLTVDKSRWQEGNVFSCSVMHEALHNHYTQKSLSLSLGKRS

SEQ ID NO: 5 - protein, 236 aa, synthetic construct
RVPITQNPCPPLKECPPCAAPDLLGGPSVFIFPPKIKDVLMISLSPMVTCVVVDVSEDDPDVQISWFVNNVEVHTAQTQTHREDYNSTLRVVSALPIQHQDWMSGKEFKCKVNNRALPSPIEKTISKPRGPVRAPQVYVLPPPAEEMTKKEFSLTCMITGFLPAEIAVDWTSNGRTEQNYKNTATVLDSDGSYFMYSKLRVQKSTWERGSLFACSVVHEGLHNHLTTKTISRSLGK

SEQ ID NO: 6 - protein, 232 aa, synthetic construct
RVPITQNLKECPPCAAPDLLGGPSVFIFPPKIKDVLMISLSPMVTCVVVDVSEDDPDVQISWFVNNVEVHTAQTQTHREDYNSTLRVVSALPIQHQDWMSGKEFKCKVNNRALPSPIEKTISKPRGPVRAPQVYVLPPPAEEMTKKEFSLTCMITGFLPAEIAVDWTSNGRTEQNYKNTATVLDSDGSYFMYSKLRVQKSTWERGSLFACSVVHEGLHNHLTTKTISRSLGK

SEQ ID NO: 7 - protein, 227 aa, synthetic construct
VPRDCGCKPCICTVPEVSSVFIFPPKPKDVLTITLTPKVTCVVVDISKDDPEVQFSWFVDDVEVHTAQTQPREEQFNSTFRSVSELPIMHQDWLNGKEFKCRVNSAAFPAPIEKTISKTKGRPKAPQVYTIPPPKEQMAKDKVSLTCMITDFFPEDITVEWQWNGQPAENYKNTQPIMNTNGSYFVYSKLNVQKSNWEAGNTFTCSVLHEGLHNHHTEKSLSHSPGK

SEQ ID NO: 8 - protein, 343 aa, synthetic construct
MMTGTIETTGNISAEKGGSIILQCHLSSTTAQVTQVNWEQQDQLLAICNADLGWHISPSFKDRVAPGPGLGLTLQSLTVNDTGEYFCIYHTYPDGTYTGRIFLEVLESSGSKSCDKTHTCPPCPAPELLGGPSVFLFPPKPKDTLMISRTPEVTCVVVDVSHEDPEVKFNWYVDGVEVHNAKTKPREEQYNSTYRVVSVLTVLHQDWLNGKEYKCKVSNKALPAPIEKTISKAKGQPREPQVYTLPPSRDELTKNQVSLTCLVKGFYPSDIAVEWESNGQPENNYKTTPPVLDSDGSFFLYSKLTVDKSRWQQGNVFSCSVMHEALHNHYTQKSLSLSPGKRS

SEQ ID NO: 9 - protein, 342 aa, synthetic construct
MMTGTIETTGNISAEKGGSIILQCHLSSTTAQVTQVNWEQQDQLLAICNADLGWHISPSFKDRVAPGPGLGLTLQSLTVNDTGEYFCIYHTYPDGTYTGRIFLEVLESSGSESKYGPPCPPCPAPEFLGGPSVFLFPPKPKDTLMISRTPEVTCVVVDVSQEDPEVQFNWYVDGVEVHNAKTKPREEQFNSTYRVVSVLTVLHQDWLNGKEYKCKVSNKGLPSSIEKTISKAKGQPREPQVYTLPPSQEEMTKNQVSLTCLVKGFYPSDIAVEWESNGQPENNYKTTPPVLDSDGSFFLYSRLTVDKSRWQEGNVFSCSVMHEALHNHYTQKSLSLSLGKRS

SEQ ID NO: 10 - protein, 343 aa, synthetic construct
TIDTKRNISAEEGGSVILQCHFSSDTAEVTQVDWKQQDQLLAIYSVDLGWHVASVFSDRVVPGPSLGLTFQSLTMNDTGEYFCTYHTYPGGIYKGRIFLKVQESSGSRVPITQNPCPPLKECPPCAAPDLLGGPSVFIFPPKIKDVLMISLSPMVTCVVVDVSEDDPDVQISWFVNNVEVHTAQTQTHREDYNSTLRVVSALPIQHQDWMSGKEFKCKVNNRALPSPIEKTISKPRGPVRAPQVYVLPPPAEEMTKKEFSLTCMITGFLPAEIAVDWTSNGRTEQNYKNTATVLDSDGSYFMYSKLRVQKSTWERGSLFACSVVHEGLHNHLTTKTISRSLGK

SEQ ID NO: 11 - protein, 339 aa, synthetic construct
TIDTKRNISAEEGGSVILQCHFSSDTAEVTQVDWKQQDQLLAIYSVDLGWHVASVFSDRVVPGPSLGLTFQSLTMNDTGEYFCTYHTYPGGIYKGRIFLKVQESSGSRVPITQNLKECPPCAAPDLLGGPSVFIFPPKIKDVLMISLSPMVTCVVVDVSEDDPDVQISWFVNNVEVHTAQTQTHREDYNSTLRVVSALPIQHQDWMSGKEFKCKVNNRALPSPIEKTISKPRGPVRAPQVYVLPPPAEEMTKKEFSLTCMITGFLPAEIAVDWTSNGRTEQNYKNTATVLDSDGSYFMYSKLRVQKSTWERGSLFACSVVHEGLHNHLTTKTISRSLGK

SEQ ID NO: 12 - protein, 334 aa, synthetic construct
TIDTKRNISAEEGGSVILQCHFSSDTAEVTQVDWKQQDQLLAIYSVDLGWHVASVFSDRVVPGPSLGLTFQSLTMNDTGEYFCTYHTYPGGIYKGRIFLKVQESSGSVPRDCGCKPCICTVPEVSSVFIFPPKPKDVLTITLTPKVTCVVVDISKDDPEVQFSWFVDDVEVHTAQTQPREEQFNSTFRSVSELPIMHQDWLNGKEFKCRVNSAAFPAPIEKTISKTKGRPKAPQVYTIPPPKEQMAKDKVSLTCMITDFFPEDITVEWQWNGQPAENYKNTQPIMNTNGSYFVYSKLNVQKSNWEAGNTFTCSVLHEGLHNHHTEKSLSHSPGK

SEQ ID NO: 13 - protein, 347 aa, synthetic construct
MMTGTIETTGNISAEKGGSIILQCHLSSTTAQVTQVNWEQQDQLLAICNADLGWHISPSFKDRVAPGPGLGLTLQSLTVNDTGEYFCIYHTYPDGTYTGRIFLEVLESSGSRVPITQNPCPPLKECPPCAAPDLLGGPSVFIFPPKIKDVLMISLSPMVTCVVVDVSEDDPDVQISWFVNNVEVHTAQTQTHREDYNSTLRVVSALPIQHQDWMSGKEFKCKVNNRALPSPIEKTISKPRGPVRAPQVYVLPPPAEEMTKKEFSLTCMITGFLPAEIAVDWTSNGRTEQNYKNTATVLDSDGSYFMYSKLRVQKSTWERGSLFACSVVHEGLHNHLTTKTISRSLGK

SEQ ID NO: 14 - protein, 343 aa, synthetic construct
MMTGTIETTGNISAEKGGSIILQCHLSSTTAQVTQVNWEQQDQLLAICNADLGWHISPSFKDRVAPGPGLGLTLQSLTVNDTGEYFCIYHTYPDGTYTGRIFLEVLESSGSRVPITQNLKECPPCAAPDLLGGPSVFIFPPKIKDVLMISLSPMVTCVVVDVSEDDPDVQISWFVNNVEVHTAQTQTHREDYNSTLRVVSALPIQHQDWMSGKEFKCKVNNRALPSPIEKTISKPRGPVRAPQVYVLPPPAEEMTKKEFSLTCMITGFLPAEIAVDWTSNGRTEQNYKNTATVLDSDGSYFMYSKLRVQKSTWERGSLFACSVVHEGLHNHLTTKTISRSLGK

SEQ ID NO: 15 - protein, 338 aa, synthetic construct
MMTGTIETTGNISAEKGGSIILQCHLSSTTAQVTQVNWEQQDQLLAICNADLGWHISPSFKDRVAPGPGLGLTLQSLTVNDTGEYFCIYHTYPDGTYTGRIFLEVLESSGSVPRDCGCKPCICTVPEVSSVFIFPPKPKDVLTITLTPKVTCVVVDISKDDPEVQFSWFVDDVEVHTAQTQPREEQFNSTFRSVSELPIMHQDWLNGKEFKCRVNSAAFPAPIEKTISKTKGRPKAPQVYTIPPPKEQMAKDKVSLTCMITDFFPEDITVEWQWNGQPAENYKNTQPIMNTNGSYFVYSKLNVQKSNWEAGNTFTCSVLHEGLHNHHTEKSLSHSPGK

SEQ ID NO: 16 - DNA, 327 bp, synthetic construct
  source 1..327: mol_type = other DNA
atgatgaccggcacaatcgagaccacaggcaacatcagcgccgagaagggcggctccatcatcctgcagtgccacctgagctccaccacagcccaggtgacacaggtgaactgggagcagcaggaccagctgctggccatctgtaatgccgatctgggctggcacatctccccttctttcaaggacagggtggcaccaggacctggactgggactgaccctgcagtccctgaccgtgaatgacacaggcgagtacttctgcatctaccacacatatcccgatggcacctatacaggcagaatctttctggaggtgctggagtctagc

SEQ ID NO: 17 - DNA, 315 bp, synthetic construct
  source 1..315: mol_type = other DNA
accatcgacacaaagaggaacatcagcgccgaggagggaggctccgtgatcctgcagtgccacttctctagcgataccgccgaggtgacacaggtggactggaagcagcaggatcagctgctggccatctacagcgtggacctgggatggcacgtggccagcgtgttttccgatagagtggtgccaggaccttccctgggactgaccttccagtctctgaccatgaacgacacaggcgagtacttttgcacctaccacacatatccaggcggcatctataagggccggatcttcctgaaggtgcaggagtcctct

SEQ ID NO: 18 - DNA, 1029 bp, synthetic construct
  source 1..1029: mol_type = other DNA
atgatgaccggcacaatcgagaccacaggcaacatcagcgccgagaagggcggctccatcatcctgcagtgccacctgagctccaccacagcccaggtgacacaggtgaactgggagcagcaggaccagctgctggccatctgtaatgccgatctgggctggcacatctccccttctttcaaggacagggtggcaccaggacctggactgggactgaccctgcagtccctgaccgtgaatgacacaggcgagtacttctgcatctaccacacatatcccgatggcacctatacaggcagaatctttctggaggtgctggagtctagcggatccaagagctgcgacaagacccacacctgccccccctgccccgcccccgagctgctgggcggccccagcgtgttcctgttcccccccaagcccaaggacaccctgatgatcagcaggacccccgaggtgacctgcgtggtggtggacgtgagccacgaggaccccgaggtgaagttcaactggtacgtggacggcgtggaggtgcacaacgccaagaccaagcccagggaggagcagtacaacagcacctacagggtggtgagcgtgctgaccgtgctgcaccaggactggctgaacggcaaggagtacaagtgcaaggtgagcaacaaggccctgcccgcccccatcgagaagaccatcagcaaggccaagggccagcccagggagccccaggtgtacaccctgccccccagcagggacgagctgaccaagaaccaggtgagcctgacctgcctggtgaagggcttctaccccagcgacatcgccgtggagtgggagagcaacggccagcccgagaacaactacaagaccaccccccccgtgctggacagcgacggcagcttcttcctgtacagcaagctgaccgtggacaagagcaggtggcagcagggcaacgtgttcagctgcagcgtgatgcacgaggccctgcacaaccactacacccagaagagcctgagcctgagccccggcaagagatct

SEQ ID NO: 19 - DNA, 1026 bp, synthetic construct
  source 1..1026: mol_type = other DNA
atgatgaccggcacaatcgagaccacaggcaacatcagcgccgagaagggcggctccatcatcctgcagtgccacctgagctccaccacagcccaggtgacacaggtgaactgggagcagcaggaccagctgctggccatctgtaatgccgatctgggctggcacatctccccttctttcaaggacagggtggcaccaggacctggactgggactgaccctgcagtccctgaccgtgaatgacacaggcgagtacttctgcatctaccacacatatcccgatggcacctatacaggcagaatctttctggaggtgctggagtctagcggatccgaaagcaaatatggcccgccgtgcccgccgtgcccggcgccggaatttctgggcggcccgagcgtgtttctgtttccgccgaaaccgaaagataccctgatgattagccgcaccccggaagtgacctgcgtggtggtggatgtgagccaggaagatccggaagtgcagtttaactggtatgtggatggcgtggaagtgcataacgcgaaaaccaaaccgcgcgaagaacagtttaacagcacctatcgcgtggtgagcgtgctgaccgtgctgcatcaggattggctgaacggcaaagaatataaatgcaaagtgagcaacaaaggcctgccgagcagcattgaaaaaaccattagcaaagcgaaaggccagccgcgcgaaccgcaggtgtataccctgccgccgagccaggaagaaatgaccaaaaaccaggtgagcctgacctgcctggtgaaaggcttttatccgagcgatattgcggtggaatgggaaagcaacggccagccggaaaacaactataaaaccaccccgccggtgctggatagcgatggcagcttttttctgtatagccgcctgaccgtggataaaagccgctggcaggaaggcaacgtgtttagctgcagcgtgatgcatgaagcgctgcataaccattatacccagaaaagcctgagcctgagcctgggcaaacgcagc

SEQ ID NO: 20 - DNA, 1029 bp, synthetic construct
  source 1..1029: mol_type = other DNA
accatcgacacaaagaggaacatcagcgccgaggagggaggctccgtgatcctgcagtgccacttctctagcgataccgccgaggtgacacaggtggactggaagcagcaggatcagctgctggccatctacagcgtggacctgggatggcacgtggccagcgtgttttccgatagagtggtgccaggaccttccctgggactgaccttccagtctctgaccatgaacgacacaggcgagtacttttgcacctaccacacatatccaggcggcatctataagggccggatcttcctgaaggtgcaggagtcctctggatcccgggtgccaatcacccagaatccttgtccccctctgaaggagtgcccaccctgtgcagccccagacctgctgggaggaccatccgtgttcatctttcctccaaagatcaaggatgtgctgatgatctctctgagccctatggtgacatgcgtggtggtggacgtgtccgaggacgatccagatgtgcagatcagctggttcgtgaacaatgtggaggtgcacaccgcccagacccagacacaccgggaggactacaactctacactgagagtggtgagcgccctgcccatccagcaccaggattggatgtccggcaaggagtttaagtgcaaggtgaacaatcgggccctgccaagccccatcgagaagaccatctccaagcctaggggaccagtgagagcaccacaggtgtacgtgctgccacctccagccgaggagatgacaaagaaggagttcagcctgacctgtatgatcacaggctttctgcctgccgagatcgccgtggactggacctccaatggcaggacagagcagaactataagaataccgccacagtgctggactctgatggcagctacttcatgtattctaagctgagggtgcagaagagcacctgggagcgcggctccctgtttgcctgctctgtggtgcacgagggcctgcacaaccacctgaccacaaagaccatctcccgctctctgggcaag

SEQ ID NO: 21 - DNA, 1017 bp, synthetic construct
  source 1..1017: mol_type = other DNA
accatcgacacaaagaggaacatcagcgccgaggagggaggctccgtgatcctgcagtgccacttctctagcgataccgccgaggtgacacaggtggactggaagcagcaggatcagctgctggccatctacagcgtggacctgggatggcacgtggccagcgtgttttccgatagagtggtgccaggaccttccctgggactgaccttccagtctctgaccatgaacgacacaggcgagtacttttgcacctaccacacatatccaggcggcatctataagggccggatcttcctgaaggtgcaggagtcctctggatcccgggtgccaatcacccagaatctgaaggagtgcccaccctgtgcagccccagacctgctgggaggaccatccgtgttcatctttcctccaaagatcaaggatgtgctgatgatctctctgagccctatggtgacatgcgtggtggtggacgtgtccgaggacgatccagatgtgcagatcagctggttcgtgaacaatgtggaggtgcacaccgcccagacccagacacaccgggaggactacaactctacactgagagtggtgagcgccctgcccatccagcaccaggattggatgtccggcaaggagtttaagtgcaaggtgaacaatcgggccctgccaagccccatcgagaagaccatctccaagcctaggggaccagtgagagcaccacaggtgtacgtgctgccacctccagccgaggagatgacaaagaaggagttcagcctgacctgtatgatcacaggctttctgcctgccgagatcgccgtggactggacctccaatggcaggacagagcagaactataagaataccgccacagtgctggactctgatggcagctacttcatgtattctaagctgagggtgcagaagagcacctgggagcgcggctccctgtttgcctgctctgtggtgcacgagggcctgcacaaccacctgaccacaaagaccatctcccgctctctgggcaag

SEQ ID NO: 22 - DNA, 1002 bp, synthetic construct
  source 1..1002: mol_type = other DNA
accatcgacacaaagaggaacatcagcgccgaggagggaggctccgtgatcctgcagtgccacttctctagcgataccgccgaggtgacacaggtggactggaagcagcaggatcagctgctggccatctacagcgtggacctgggatggcacgtggccagcgtgttttccgatagagtggtgccaggaccttccctgggactgaccttccagtctctgaccatgaacgacacaggcgagtacttttgcacctaccacacatatccaggcggcatctataagggccggatcttcctgaaggtgcaggagtcctctggatccgtgccacgggactgcggctgtaagccctgcatctgtacagtgcctgaggtgagctccgtgttcatctttccccctaagcctaaggacgtgctgaccatcacactgaccccaaaggtgacctgcgtggtggtggatatcagcaaggacgatcccgaggtgcagttctcctggtttgtggacgatgtggaggtgcacacagcacagacccagccaagggaggagcagttcaattccacctttagatctgtgagcgagctgcctatcatgcaccaggactggctgaatggcaaggagttcaagtgcagggtgaactccgccgcctttccagcccccatcgagaagacaatctctaagaccaagggccgccctaaggccccacaggtgtacacaatcccaccccctaaggagcagatggccaaggataaggtgagcctgacatgtatgatcaccgacttctttcctgaggatatcaccgtggagtggcagtggaacggccagccagccgagaactataagaatacacagcccatcatgaacaccaatggctcctacttcgtgtattctaagctgaacgtgcagaagtctaattgggaggccggcaacaccttcacctgtagcgtgctgcacgagggcctgcacaatcaccacacagagaagtccctgtctcacagccccggcaag

SEQ ID NO: 23 - DNA, 1041 bp, synthetic construct
  source 1..1041: mol_type = other DNA
atgatgaccggcacaatcgagaccacaggcaacatctccgccgagaagggcggctctatcatcctgcagtgccacctgtctagcaccacagcccaggtgacccaggtgaactgggagcagcaggaccagctgctggccatctgtaatgccgatctgggctggcacatcagcccatccttcaaggacagggtggcaccaggacctggactgggactgaccctgcagagcctgaccgtgaacgacacaggcgagtacttctgcatctaccacacatatcccgatggcacctatacaggcaggatctttctggaggtgctggagtcctctggctcccgcgtgcccatcacccagaatccttgtccccctctgaaggagtgcccaccctgtgcagccccagacctgctgggaggaccaagcgtgttcatctttcctccaaagatcaaggatgtgctgatgatctctctgagccctatggtgacctgcgtggtggtggacgtgagcgaggacgatccagatgtgcagatcagctggttcgtgaacaatgtggaggtgcacaccgcccagacccagacacacagggaggactacaacagcacactgagggtggtgtccgccctgcctatccagcaccaggattggatgtccggcaaggagtttaagtgcaaggtgaacaatagagccctgccatctcccatcgagaagaccatcagcaagcctaggggaccagtgagagcaccacaggtgtacgtgctgccacctccagccgaggagatgacaaagaaggagttctctctgacctgtatgatcacaggctttctgcctgccgagatcgccgtggactggaccagcaatggcaggacagagcagaactataagaataccgccacagtgctggacagcgatggctcctacttcatgtattccaagctgcgggtgcagaagtctacctgggagagaggctctctgtttgcctgtagcgtggtgcacgagggcctgcacaaccacctgaccacaaagaccatctcccgctctctgggcaag

SEQ ID NO: 24 - DNA, 1029 bp, synthetic construct
  source 1..1029: mol_type = other DNA
atgatgaccggcacaatcgagaccacaggcaacatctccgccgagaagggcggctctatcatcctgcagtgccacctgtctagcaccacagcccaggtgacccaggtgaactgggagcagcaggaccagctgctggccatctgtaatgccgatctgggctggcacatcagcccatccttcaaggacagggtggcaccaggacctggactgggactgaccctgcagagcctgaccgtgaacgacacaggcgagtacttctgcatctaccacacatatcccgatggcacctatacaggcaggatctttctggaggtgctggagtcctctggctcccgcgtgcccatcacccagaatctgaaggagtgcccaccctgtgcagccccagacctgctgggaggaccaagcgtgttcatctttcctccaaagatcaaggatgtgctgatgatctctctgagccctatggtgacctgcgtggtggtggacgtgagcgaggacgatccagatgtgcagatcagctggttcgtgaacaatgtggaggtgcacaccgcccagacccagacacacagggaggactacaacagcacactgagggtggtgtccgccctgcctatccagcaccaggattggatgtccggcaaggagtttaagtgcaaggtgaacaatagagccctgccatctcccatcgagaagaccatcagcaagcctaggggaccagtgagagcaccacaggtgtacgtgctgccacctccagccgaggagatgacaaagaaggagttctctctgacctgtatgatcacaggctttctgcctgccgagatcgccgtggactggaccagcaatggcaggacagagcagaactataagaataccgccacagtgctggacagcgatggctcctacttcatgtattccaagctgcgggtgcagaagtctacctgggagagaggctctctgtttgcctgtagcgtggtgcacgagggcctgcacaaccacctgaccacaaagaccatctcccgctctctgggcaag

SEQ ID NO: 25 - DNA, 1014 bp, synthetic construct
  source 1..1014: mol_type = other DNA
atgatgaccggcacaatcgagaccacaggcaacatctccgccgagaagggcggctctatcatcctgcagtgccacctgtctagcaccacagcccaggtgacccaggtgaactgggagcagcaggaccagctgctggccatctgtaatgccgatctgggctggcacatcagcccatccttcaaggacagggtggcaccaggacctggactgggactgaccctgcagagcctgaccgtgaacgacacaggcgagtacttctgcatctaccacacatatcccgatggcacctatacaggcaggatctttctggaggtgctggagtcctctggatccgtgccacgggactgcggctgtaagccctgcatctgtacagtgcctgaggtgagctccgtgttcatctttccccctaagcctaaggacgtgctgaccatcacactgaccccaaaggtgacctgcgtggtggtggatatcagcaaggacgatcccgaggtgcagttctcctggtttgtggacgatgtggaggtgcacacagcacagacccagccaagggaggagcagttcaattccacctttaggtccgtgagcgagctgcctatcatgcaccaggactggctgaatggcaaggagttcaagtgcagggtgaactccgccgcctttccagcccccatcgagaagacaatctctaagaccaagggccgccctaaggccccacaggtgtacacaatcccaccccctaaggagcagatggccaaggataaggtgagcctgacatgtatgatcaccgacttctttcctgaggatatcaccgtggagtggcagtggaacggccagccagccgagaactataagaatacacagcccatcatgaacaccaatggctcctacttcgtgtattctaagctgaacgtgcagaagtctaattgggaggccggcaacaccttcacctgtagcgtgctgcacgagggcctgcacaatcaccacacagagaagtccctgtctcacagccccggcaag

SEQ ID NO: 26 - protein, 21 aa, Homo sapiens
MRWCLLLIWAQGLRQAPLASG

SEQ ID NO: 27 - protein, 24 aa, Homo sapiens
MPMGSLQPLATLYLLGMLVASVLA

SEQ ID NO: 28 - protein, 19 aa, Homo sapiens
MTRLTVLALLAGLLASSRA

SEQ ID NO: 29 - DNA, 384 bp, synthetic construct
  source 1..384: mol_type = other DNA
atgacccggctgaccgtgctggccctgctggccggcctgctggccagcagccgggccatgatgaccggcacaatcgagaccacaggcaacatcagcgccgagaagggcggctccatcatcctgcagtgccacctgagctccaccacagcccaggtgacacaggtgaactgggagcagcaggaccagctgctggccatctgtaatgccgatctgggctggcacatctccccttctttcaaggacagggtggcaccaggacctggactgggactgaccctgcagtccctgaccgtgaatgacacaggcgagtacttctgcatctaccacacatatcccgatggcacctatacaggcagaatctttctggaggtgctggagtctagc

SEQ ID NO: 30 - DNA, 372 bp, synthetic construct
  source 1..372: mol_type = other DNA
atgacccggctgacagtgctggccctgctggccggactgctggccagctccagggcaaccatcgacacaaagaggaacatcagcgccgaggagggaggctccgtgatcctgcagtgccacttctctagcgataccgccgaggtgacacaggtggactggaagcagcaggatcagctgctggccatctacagcgtggacctgggatggcacgtggccagcgtgttttccgatagagtggtgccaggaccttccctgggactgaccttccagtctctgaccatgaacgacacaggcgagtacttttgcacctaccacacatatccaggcggcatctataagggccggatcttcctgaaggtgcaggagtcctct

SEQ ID NO: 31 - DNA, 1086 bp, synthetic construct
  source 1..1086: mol_type = other DNA
atgacccggctgaccgtgctggccctgctggccggcctgctggccagcagccgggccatgatgaccggcacaatcgagaccacaggcaacatcagcgccgagaagggcggctccatcatcctgcagtgccacctgagctccaccacagcccaggtgacacaggtgaactgggagcagcaggaccagctgctggccatctgtaatgccgatctgggctggcacatctccccttctttcaaggacagggtggcaccaggacctggactgggactgaccctgcagtccctgaccgtgaatgacacaggcgagtacttctgcatctaccacacatatcccgatggcacctatacaggcagaatctttctggaggtgctggagtctagcggatccaagagctgcgacaagacccacacctgccccccctgccccgcccccgagctgctgggcggccccagcgtgttcctgttcccccccaagcccaaggacaccctgatgatcagcaggacccccgaggtgacctgcgtggtggtggacgtgagccacgaggaccccgaggtgaagttcaactggtacgtggacggcgtggaggtgcacaacgccaagaccaagcccagggaggagcagtacaacagcacctacagggtggtgagcgtgctgaccgtgctgcaccaggactggctgaacggcaaggagtacaagtgcaaggtgagcaacaaggccctgcccgcccccatcgagaagaccatcagcaaggccaagggccagcccagggagccccaggtgtacaccctgccccccagcagggacgagctgaccaagaaccaggtgagcctgacctgcctggtgaagggcttctaccccagcgacatcgccgtggagtgggagagcaacggccagcccgagaacaactacaagaccaccccccccgtgctggacagcgacggcagcttcttcctgtacagcaagctgaccgtggacaagagcaggtggcagcagggcaacgtgttcagctgcagcgtgatgcacgaggccctgcacaaccactacacccagaagagcctgagcctgagccccggcaagagatct

SEQ ID NO: 32 - DNA, 1083 bp, synthetic construct
  source 1..1083: mol_type = other DNA
atgacccggctgaccgtgctggccctgctggccggcctgctggccagcagccgggccatgatgaccggcacaatcgagaccacaggcaacatcagcgccgagaagggcggctccatcatcctgcagtgccacctgagctccaccacagcccaggtgacacaggtgaactgggagcagcaggaccagctgctggccatctgtaatgccgatctgggctggcacatctccccttctttcaaggacagggtggcaccaggacctggactgggactgaccctgcagtccctgaccgtgaatgacacaggcgagtacttctgcatctaccacacatatcccgatggcacctatacaggcagaatctttctggaggtgctggagtctagcggatccgaaagcaaatatggcccgccgtgcccgccgtgcccggcgccggaatttctgggcggcccgagcgtgtttctgtttccgccgaaaccgaaagataccctgatgattagccgcaccccggaagtgacctgcgtggtggtggatgtgagccaggaagatccggaagtgcagtttaactggtatgtggatggcgtggaagtgcataacgcgaaaaccaaaccgcgcgaagaacagtttaacagcacctatcgcgtggtgagcgtgctgaccgtgctgcatcaggattggctgaacggcaaagaatataaatgcaaagtgagcaacaaaggcctgccgagcagcattgaaaaaaccattagcaaagcgaaaggccagccgcgcgaaccgcaggtgtataccctgccgccgagccaggaagaaatgaccaaaaaccaggtgagcctgacctgcctggtgaaaggcttttatccgagcgatattgcggtggaatgggaaagcaacggccagccggaaaacaactataaaaccaccccgccggtgctggatagcgatggcagcttttttctgtatagccgcctgaccgtggataaaagccgctggcaggaaggcaacgtgtttagctgcagcgtgatgcatgaagcgctgcataaccattatacccagaaaagcctgagcctgagcctgggcaaacgcagc

SEQ ID NO: 33 - DNA, 1086 bp, synthetic construct
  source 1..1086: mol_type = other DNA
atgacccggctgacagtgctggccctgctggccggactgctggccagctccagggcaaccatcgacacaaagaggaacatcagcgccgaggagggaggctccgtgatcctgcagtgccacttctctagcgataccgccgaggtgacacaggtggactggaagcagcaggatcagctgctggccatctacagcgtggacctgggatggcacgtggccagcgtgttttccgatagagtggtgccaggaccttccctgggactgaccttccagtctctgaccatgaacgacacaggcgagtacttttgcacctaccacacatatccaggcggcatctataagggccggatcttcctgaaggtgcaggagtcctctggatcccgggtgccaatcacccagaatccttgtccccctctgaaggagtgcccaccctgtgcagccccagacctgctgggaggaccatccgtgttcatctttcctccaaagatcaaggatgtgctgatgatctctctgagccctatggtgacatgcgtggtggtggacgtgtccgaggacgatccagatgtgcagatcagctggttcgtgaacaatgtggaggtgcacaccgcccagacccagacacaccgggaggactacaactctacactgagagtggtgagcgccctgcccatccagcaccaggattggatgtccggcaaggagtttaagtgcaaggtgaacaatcgggccctgccaagccccatcgagaagaccatctccaagcctaggggaccagtgagagcaccacaggtgtacgtgctgccacctccagccgaggagatgacaaagaaggagttcagcctgacctgtatgatcacaggctttctgcctgccgagatcgccgtggactggacctccaatggcaggacagagcagaactataagaataccgccacagtgctggactctgatggcagctacttcatgtattctaagctgagggtgcagaagagcacctgggagcgcggctccctgtttgcctgctctgtggtgcacgagggcctgcacaaccacctgaccacaaagaccatctcccgctctctgggcaag

SEQ ID NO: 34 - DNA, 1074 bp, synthetic construct
  source 1..1074: mol_type = other DNA
atgacccggctgacagtgctggccctgctggccggactgctggccagctccagggcaaccatcgacacaaagaggaacatcagcgccgaggagggaggctccgtgatcctgcagtgccacttctctagcgataccgccgaggtgacacaggtggactggaagcagcaggatcagctgctggccatctacagcgtggacctgggatggcacgtggccagcgtgttttccgatagagtggtgccaggaccttccctgggactgaccttccagtctctgaccatgaacgacacaggcgagtacttttgcacctaccacacatatccaggcggcatctataagggccggatcttcctgaaggtgcaggagtcctctggatcccgggtgccaatcacccagaatctgaaggagtgcccaccctgtgcagccccagacctgctgggaggaccatccgtgttcatctttcctccaaagatcaaggatgtgctgatgatctctctgagccctatggtgacatgcgtggtggtggacgtgtccgaggacgatccagatgtgcagatcagctggttcgtgaacaatgtggaggtgcacaccgcccagacccagacacaccgggaggactacaactctacactgagagtggtgagcgccctgcccatccagcaccaggattggatgtccggcaaggagtttaagtgcaaggtgaacaatcgggccctgccaagccccatcgagaagaccatctccaagcctaggggaccagtgagagcaccacaggtgtacgtgctgccacctccagccgaggagatgacaaagaaggagttcagcctgacctgtatgatcacaggctttctgcctgccgagatcgccgtggactggacctccaatggcaggacagagcagaactataagaataccgccacagtgctggactctgatggcagctacttcatgtattctaagctgagggtgcagaagagcacctgggagcgcggctccctgtttgcctgctctgtggtgcacgagggcctgcacaaccacctgaccacaaagaccatctcccgctctctgggcaag

SEQ ID NO: 35 - DNA, 1059 bp, synthetic construct
  source 1..1059: mol_type = other DNA
atgacccggctgacagtgctggccctgctggccggactgctggccagctccagggcaaccatcgacacaaagaggaacatcagcgccgaggagggaggctccgtgatcctgcagtgccacttctctagcgataccgccgaggtgacacaggtggactggaagcagcaggatcagctgctggccatctacagcgtggacctgggatggcacgtggccagcgtgttttccgatagagtggtgccaggaccttccctgggactgaccttccagtctctgaccatgaacgacacaggcgagtacttttgcacctaccacacatatccaggcggcatctataagggccggatcttcctgaaggtgcaggagtcctctggatccgtgccacgggactgcggctgtaagccctgcatctgtacagtgcctgaggtgagctccgtgttcatctttccccctaagcctaaggacgtgctgaccatcacactgaccccaaaggtgacctgcgtggtggtggatatcagcaaggacgatcccgaggtgcagttctcctggtttgtggacgatgtggaggtgcacacagcacagacccagccaagggaggagcagttcaattccacctttagatctgtgagcgagctgcctatcatgcaccaggactggctgaatggcaaggagttcaagtgcagggtgaactccgccgcctttccagcccccatcgagaagacaatctctaagaccaagggccgccctaaggccccacaggtgtacacaatcccaccccctaaggagcagatggccaaggataaggtgagcctgacatgtatgatcaccgacttctttcctgaggatatcaccgtggagtggcagtggaacggccagccagccgagaactataagaatacacagcccatcatgaacaccaatggctcctacttcgtgtattctaagctgaacgtgcagaagtctaattgggaggccggcaacaccttcacctgtagcgtgctgcacgagggcctgcacaatcaccacacagagaagtccctgtctcacagccccggcaag

SEQ ID NO: 36 - DNA, 1098 bp, synthetic construct
  source 1..1098: mol_type = other DNA
atgacccggctgacagtgctggccctgctggccggactgctggccagctccagagccatgatgaccggcacaatcgagaccacaggcaacatctccgccgagaagggcggctctatcatcctgcagtgccacctgtctagcaccacagcccaggtgacccaggtgaactgggagcagcaggaccagctgctggccatctgtaatgccgatctgggctggcacatcagcccatccttcaaggacagggtggcaccaggacctggactgggactgaccctgcagagcctgaccgtgaacgacacaggcgagtacttctgcatctaccacacatatcccgatggcacctatacaggcaggatctttctggaggtgctggagtcctctggctcccgcgtgcccatcacccagaatccttgtccccctctgaaggagtgcccaccctgtgcagccccagacctgctgggaggaccaagcgtgttcatctttcctccaaagatcaaggatgtgctgatgatctctctgagccctatggtgacctgcgtggtggtggacgtgagcgaggacgatccagatgtgcagatcagctggttcgtgaacaatgtggaggtgcacaccgcccagacccagacacacagggaggactacaacagcacactgagggtggtgtccgccctgcctatccagcaccaggattggatgtccggcaaggagtttaagtgcaaggtgaacaatagagccctgccatctcccatcgagaagaccatcagcaagcctaggggaccagtgagagcaccacaggtgtacgtgctgccacctccagccgaggagatgacaaagaaggagttctctctgacctgtatgatcacaggctttctgcctgccgagatcgccgtggactggaccagcaatggcaggacagagcagaactataagaataccgccacagtgctggacagcgatggctcctacttcatgtattccaagctgcgggtgcagaagtctacctgggagagaggctctctgtttgcctgtagcgtggtgcacgagggcctgcacaaccacctgaccacaaagaccatctcccgctctctgggcaag

SEQ ID NO: 37 - DNA, 1086 bp, synthetic construct
  source 1..1086: mol_type = other DNA
atgacccggctgacagtgctggccctgctggccggactgctggccagctccagagccatgatgaccggcacaatcgagaccacaggcaacatctccgccgagaagggcggctctatcatcctgcagtgccacctgtctagcaccacagcccaggtgacccaggtgaactgggagcagcaggaccagctgctggccatctgtaatgccgatctgggctggcacatcagcccatccttcaaggacagggtggcaccaggacctggactgggactgaccctgcagagcctgaccgtgaacgacacaggcgagtacttctgcatctaccacacatatcccgatggcacctatacaggcaggatctttctggaggtgctggagtcctctggctcccgcgtgcccatcacccagaatctgaaggagtgcccaccctgtgcagccccagacctgctgggaggaccaagcgtgttcatctttcctccaaagatcaaggatgtgctgatgatctctctgagccctatggtgacctgcgtggtggtggacgtgagcgaggacgatccagatgtgcagatcagctggttcgtgaacaatgtggaggtgcacaccgcccagacccagacacacagggaggactacaacagcacactgagggtggtgtccgccctgcctatccagcaccaggattggatgtccggcaaggagtttaagtgcaaggtgaacaatagagccctgccatctcccatcgagaagaccatcagcaagcctaggggaccagtgagagcaccacaggtgtacgtgctgccacctccagccgaggagatgacaaagaaggagttctctctgacctgtatgatcacaggctttctgcctgccgagatcgccgtggactggaccagcaatggcaggacagagcagaactataagaataccgccacagtgctggacagcgatggctcctacttcatgtattccaagctgcgggtgcagaagtctacctgggagagaggctctctgtttgcctgtagcgtggtgcacgagggcctgcacaaccacctgaccacaaagaccatctcccgctctctgggcaag

SEQ ID NO: 38 - DNA, 1071 bp, synthetic construct
  source 1..1071: mol_type = other DNA
atgacccggctgacagtgctggccctgctggccggactgctggccagctccagagccatgatgaccggcacaatcgagaccacaggcaacatctccgccgagaagggcggctctatcatcctgcagtgccacctgtctagcaccacagcccaggtgacccaggtgaactgggagcagcaggaccagctgctggccatctgtaatgccgatctgggctggcacatcagcccatccttcaaggacagggtggcaccaggacctggactgggactgaccctgcagagcctgaccgtgaacgacacaggcgagtacttctgcatctaccacacatatcccgatggcacctatacaggcaggatctttctggaggtgctggagtcctctggatccgtgccacgggactgcggctgtaagccctgcatctgtacagtgcctgaggtgagctccgtgttcatctttccccctaagcctaaggacgtgctgaccatcacactgaccccaaaggtgacctgcgtggtggtggatatcagcaaggacgatcccgaggtgcagttctcctggtttgtggacgatgtggaggtgcacacagcacagacccagccaagggaggagcagttcaattccacctttaggtccgtgagcgagctgcctatcatgcaccaggactggctgaatggcaaggagttcaagtgcagggtgaactccgccgcctttccagcccccatcgagaagacaatctctaagaccaagggccgccctaaggccccacaggtgtacacaatcccaccccctaaggagcagatggccaaggataaggtgagcctgacatgtatgatcaccgacttctttcctgaggatatcaccgtggagtggcagtggaacggccagccagccgagaactataagaatacacagcccatcatgaacaccaatggctcctacttcgtgtattctaagctgaacgtgcagaagtctaattgggaggccggcaacaccttcacctgtagcgtgctgcacgagggcctgcacaatcaccacacagagaagtccctgtctcacagccccggcaag

SEQ ID NO: 39 - protein, 123 aa, synthetic construct
GMMTGTIETTGNISAEKGGSIILQCHLSSTTAQVTQVNWEQQDQLLAICNADLGWHISPSFKDRVAPGPGLGLTLQSLTVNDTGEYFCIYHTYPDGTYTGRIFLEVLESSVAEHGARFQIPLE

SEQ ID NO: 40 - protein, 11 aa, synthetic construct
NISAEKGGSII

SEQ ID NO: 41 - protein, 11 aa, synthetic construct
NISAEEGGSVI

SEQ ID NO: 42 - DNA, 21 bp, synthetic construct
  source 1..21: mol_type = other DNA
cgcaaatgggcggtaggcgtg

SEQ ID NO: 43 - DNA, 21 bp, synthetic construct
  source 1..21: mol_type = other DNA
catagcgtaaaaggagcaaca

SEQ ID NO: 44 - protein, 6 aa, synthetic construct
HHHHHH

SEQ ID NO: 45 - protein, 4 aa, synthetic construct
PCPP